European Patent Specification EP 3 701 967 B1, published July 30, 2025. Title: Use of Jack bean Lectin for increasing the abundance of hematopoietic stem cells and progenitor cells in bone marrow and/or epidermal stem cells in skin in vivo. Applicant: The Secretary DEPARTMENT OF ATOMIC ENERGY [IN/IN], Mumbai -400001, Maharastra (IN). The sequence listing filed with the application follows.

SEQUENCE LISTING (1 sequence)

SEQ ID NO: 1 - protein, 235 aa, Jack Bean Lectin
ADTIVAVELDTYPNTDIGDPSYPHIGIDIKSVRSKKTAKWNMQNGKVGTAHIIYNSVDKRLSAVVSYPNADSATVSYDVDLDNVLPEWVRVGLSASTGLYKETNTILSWSFTSKLKSNTHETNALHFMNQFSKDQKDLILQGDATTGTDGNLELTRVSSNGSPQGSSVGRALFYAPVHIWESSAVVASFEATFTFLIKSPDSHPADGIAFFISNIDSSIPSGSTGRLLGLFPDAN